European Patent Application EP 4 814 012 A1, published September 30, 2026. Title: 抗IL-4Rα抗体或其抗原结合片段及其双特异性抗体和应用. Applicant: 联邦生物科技（珠海横琴）有限公司. The sequence listing filed with the application follows.

SEQUENCE LISTING (60 sequences)

SEQ ID NO: 1 - protein, 10 aa, Artificial Sequence
GYTFTTYYIY

SEQ ID NO: 2 - protein, 17 aa, Artificial Sequence
GSNPSTGGTLDNEKFKT

SEQ ID NO: 3 - protein, 9 aa, Artificial Sequence
SGRYAPFTY

SEQ ID NO: 4 - protein, 11 aa, Artificial Sequence
KASQDVSTSVA

SEQ ID NO: 5 - protein, 7 aa, Artificial Sequence
SASYRFT

SEQ ID NO: 6 - protein, 9 aa, Artificial Sequence
QHYSTTPFT

SEQ ID NO: 7 - protein, 17 aa, Artificial Sequence
GSNPSTGGTLENEKFKT

SEQ ID NO: 8 - protein, 9 aa, Artificial Sequence
VHYSTTPFT

SEQ ID NO: 9 - protein, 9 aa, Artificial Sequence
SGRYATFTY

SEQ ID NO: 10 - protein, 17 aa, Artificial Sequence
GSNPSTGGTLFNEKFKT

SEQ ID NO: 11 - protein, 9 aa, Artificial Sequence
QQYSTTPFT

SEQ ID NO: 12 - protein, 10 aa, Artificial Sequence
GFTFSSYYMS

SEQ ID NO: 13 - protein, 17 aa, Artificial Sequence
AINSNGGSTYSPDTVKG

SEQ ID NO: 14 - protein, 14 aa, Artificial Sequence
RSLLGNHRDWYFDV

SEQ ID NO: 15 - protein, 11 aa, Artificial Sequence
RASENIYSYLA

SEQ ID NO: 16 - protein, 7 aa, Artificial Sequence
NAKTLAD

SEQ ID NO: 17 - protein, 9 aa, Artificial Sequence
LHHYGTPLT

SEQ ID NO: 18 - protein, 118 aa, Artificial Sequence
QVQLQQPGAELVKPGASMKLSCKASGYTFTTYYIYWVKQRPGQGLEWIGGSNPSTGGTLFNEKFKTKATLTVDKYSSTAYMELSSLTFEDSAVYFCTRSGRYAPFTYWGQGTLVTVSA

SEQ ID NO: 19 - protein, 107 aa, Artificial Sequence
DIVMTQSHKVLSTSVGDRVIITCKASQDVSTSVAWYQQRPGHSPKLLIYSASYRFTGVPDRFTGSGSGTDFTFTISSVQAEDLAVYNCQQYSTTPFTFGSGTKLEIK

SEQ ID NO: 20 - protein, 123 aa, Artificial Sequence
DVKLVESGGGLVKLGGSLKLSCAASGFTFSSYYMSWVRQTPEKRLELVAAINSNGGSTYSPDTVKGRFTISRDNAKNTLYLQMSSLKSEDTALYYCARRSLLGNHRDWYFDVWGAGTTVTVSS

SEQ ID NO: 21 - protein, 107 aa, Artificial Sequence
DIQMTQSPASLSASVGETVTITCRASENIYSYLAWYQQKQGKSPQLLVYNAKTLADGVPSRFSGSGSGTQFSLKINTLQPEDFGSYYCLHHYGTPLTFGAGTKLELK

SEQ ID NO: 22 - protein, 118 aa, Artificial Sequence
QVQLVQSGAEVKKPGASVKVSCKASGYTFTTYYIYWVRQAPGQGLEWMGGSNPSTGGTLFNEKFKTRVTMTRDTSTSTVYMELSSLRSEDTAVYYCARSGRYAPFTYWGQGTLVTVSS

SEQ ID NO: 23 - protein, 107 aa, Artificial Sequence
DIQMTQSPSSLSASVGDRVTITCKASQDVSTSVAWYQQKPGKAPKLLIYSASYRFTGVPSRFSGSGSGTDFTLTISSLQPEDFATYYCQQYSTTPFTFGQGTKLEIK

SEQ ID NO: 24 - protein, 123 aa, Artificial Sequence
EVQLVESGGGLVKPGGSLRLSCAASGFTFSSYYMSWVRQAPGKGLEWVSAINSNGGSTYSPDTVKGRFTISRDNAKNSLYLQMNSLRAEDTAVYYCARRSLLGNHRDWYFDVWGQGTTVTVSS

SEQ ID NO: 25 - protein, 107 aa, Artificial Sequence
DIQMTQSPSSLSASVGDRVTITCRASENIYSYLAWYQQKPGKAPKLLIYNAKTLADGVPSRFSGSGSGTDFTLTISSLQPEDFATYYCLHHYGTPLTFGQGTKLEIK

SEQ ID NO: 26 - protein, 118 aa, Artificial Sequence
QVQLVQSGAEVKKPGASVKVSCKASGYTFTTYYIYWVRQAPGQGLEWMGGSNPSTGGTLFNEKFKTRVTMTVDKSTSTAYMELSSLRSEDTAVYYCTRSGRYAPFTYWGQGTLVTVSS

SEQ ID NO: 27 - protein, 107 aa, Artificial Sequence
DIQMTQSPSSLSASVGDRVTITCKASQDVSTSVAWYQQKPGKAPKLLIYSASYRFTGVPSRFSGSGSGTDFTFTISSLQPEDFATYYCQQYSTTPFTFGQGTKLEIK

SEQ ID NO: 28 - protein, 118 aa, Artificial Sequence
QVQLVQSGAEVKKPGASVKVSCKASGYTFTTYYIYWVRQAPGQGLEWMGGSNPSTGGTLDNEKFKTRVTMTVDKSTSTAYMELSSLRSEDTAVYYCTRSGRYAPFTYWGQGTLVTVSS

SEQ ID NO: 29 - protein, 107 aa, Artificial Sequence
DIQMTQSPSSLSASVGDRVTITCKASQDVSTSVAWYQQKPGKAPKLLIYSASYRFTGVPSRFSGSGSGTDFTFTISSLQPEDFATYYCQHYSTTPFTFGQGTKLEIK

SEQ ID NO: 30 - protein, 118 aa, Artificial Sequence
QVQLVQSGAEVKKPGASVKVSCKASGYTFTTYYIYWVRQAPGQGLEWMGGSNPSTGGTLENEKFKTRVTMTVDKSTSTAYMELSSLRSEDTAVYYCTRSGRYAPFTYWGQGTLVTVSS

SEQ ID NO: 31 - protein, 107 aa, Artificial Sequence
DIQMTQSPSSLSASVGDRVTITCKASQDVSTSVAWYQQKPGKAPKLLIYSASYRFTGVPSRFSGSGSGTDFTFTISSLQPEDFATYYCVHYSTTPFTFGQGTKLEIK

SEQ ID NO: 32 - protein, 118 aa, Artificial Sequence
QVQLVQSGAEVKKPGASVKVSCKASGYTFTTYYIYWVRQAPGQGLEWMGGSNPSTGGTLENEKFKTRVTMTVDKSTSTAYMELSSLRSEDTAVYYCTRSGRYATFTYWGQGTLVTVSS

SEQ ID NO: 33 - protein, 107 aa, Artificial Sequence; identical to SEQ ID NO: 31

SEQ ID NO: 34 - protein, 122 aa, Artificial Sequence
QMQLVESGGGVVQPGRSLRLSCAASGFTFRTYGMHWVRQAPGKGLEWVAVIWYDGSNKHYADSVKGRFTITRDNSKNTLNLQMNSLRAEDTAVYYCARAPQWELVHEAFDIWGQGTMVTVSS

SEQ ID NO: 35 - protein, 326 aa, Artificial Sequence
ASTKGPSVFPLAPCSRSTSESTAALGCLVKDYFPEPVTVSWNSGALTSGVHTFPAVLQSSGLYSLSSVVTVPSSNFGTQTYTCNVDHKPSNTKVDKTVERKCCVECPPCPAPPVAGPSVFLFPPKPKDTLMISRTPEVTCVVVDVSHEDPEVQFNWYVDGVEVHNAKTKPREEQFNSTFRVVSVLTVVHQDWLNGKEYKCKVSNKGLPAPIEKTISKTKGQPREPQVYTLPPSREEMTKNQVSLTCLVKGFYPSDIAVEWESNGQPENNYKTTPPMLDSDGSFFLYSKLTVDKSRWQQGNVFSCSVMHEALHNHYTQKSLSLSPGK

SEQ ID NO: 36 - protein, 108 aa, Artificial Sequence
SYVLTQPPSVSVAPGQTARITCGGNNLGSKSVHWYQQKPGQAPVLVVYDDSDRPSWIPERFSGSNSGNTATLTISRGEAGDEADYYCQVWDSSSDHVVFGGGTKLTVL

SEQ ID NO: 37 - protein, 106 aa, Artificial Sequence
GQPKAAPSVTLFPPSSEELQANKATLVCLISDFYPGAVTVAWKADSSPVKAGVETTTPSKQSNNKYAASSYLSLTPEQWKSHRSYSCQVTHEGSTVEKTVAPTECS

SEQ ID NO: 38 - protein, 452 aa, Artificial Sequence
EVQLVESGGGLEQPGGSLRLSCAGSGFTFRDYAMTWVRQAPGKGLEWVSSISGSGGNTYYADSVKGRFTISRDNSKNTLYLQMNSLRAEDTAVYYCAKDRLSITIRPRYYGLDVWGQGTTVTVSSASTKGPSVFPLAPCSRSTSESTAALGCLVKDYFPEPVTVSWNSGALTSGVHTFPAVLQSSGLYSLSSVVTVPSSSLGTKTYTCNVDHKPSNTKVDKRVESKYGPPCPPCPAPEFLGGPSVFLFPPKPKDTLMISRTPEVTCVVVDVSQEDPEVQFNWYVDGVEVHNAKTKPREEQFNSTYRVVSVLTVLHQDWLNGKEYKCKVSNKGLPSSIEKTISKAKGQPREPQVYTLPPSQEEMTKNQVSLTCLVKGFYPSDIAVEWESNGQPENNYKTTPPVLDSDGSFFLYSRLTVDKSRWQEGNVFSCSVMHEALHNHYTQKSLSLSLGK

SEQ ID NO: 39 - protein, 219 aa, Artificial Sequence
DIVMTQSPLSLPVTPGEPASISCRSSQSLLYSIGYNYLDWYLQKSGQSPQLLIYLGSNRASGVPDRFSGSGSGTDFTLKISRVEAEDVGFYYCMQALQTPYTFGQGTKLEIKRTVAAPSVFIFPPSDEQLKSGTASVVCLLNNFYPREAKVQWKVDNALQSGNSQESVTEQDSKDSTYSLSSTLTLSKADYEKHKVYACEVTHQGLSSPVTKSFNRGEC

SEQ ID NO: 40 - protein, 327 aa, Artificial Sequence
ASTKGPSVFPLAPCSRSTSESTAALGCLVKDYFPEPVTVSWNSGALTSGVHTFPAVLQSSGLYSLSSVVTVPSSSLGTKTYTCNVDHKPSNTKVDKRVESKYGPPCPPCPAPEFLGGPSVFLFPPKPKDTLMISRTPEVTCVVVDVSQEDPEVQFNWYVDGVEVHNAKTKPREEQFNSTYRVVSVLTVLHQDWLNGKEYKCKVSNKGLPSSIEKTISKAKGQPREPQVYTLPPSQEEMTKNQVSLTCLVKGFYPSDIAVEWESNGQPENNYKTTPPVLDSDGSFFLYSRLTVDKSRWQEGNVFSCSVMHEALHNHYTQKSLSLSLGK

SEQ ID NO: 41 - protein, 107 aa, Artificial Sequence [sequence omitted]

SEQ ID NO: 42 - protein, 122 aa, Artificial Sequence
QMQLVESGGGVVQPGRSLRLSCAASGFTFRTYGMHWVRQAPGKCLEWVAVIWYDGSNKHYADSVKGRFTITRDNSKNTLNLQMNSLRAEDTAVYYCARAPQWELVHEAFDIWGQGTMVTVSS

SEQ ID NO: 43 - protein, 108 aa, Artificial Sequence
SYVLTQPPSVSVAPGQTARITCGGNNLGSKSVHWYQQKPGQAPVLVVYDDSDRPSWIPERFSGSNSGNTATLTISRGEAGDEADYYCQVWDSSSDHVVFGCGTKLTVL

SEQ ID NO: 44 - protein, 118 aa, Artificial Sequence
QVQLVQSGAEVKKPGASVKVSCKASGYTFTTYYIYWVRQAPGQCLEWMGGSNPSTGGTLDNEKFKTRVTMTVDKSTSTAYMELSSLRSEDTAVYYCTRSGRYAPFTYWGCGTLVTVSS

SEQ ID NO: 45 - protein, 107 aa, Artificial Sequence
DIQMTQSPSSLSASVGDRVTITCKASQDVSTSVAWYQQKPGKAPKLLIYSASYRFTGVPSRFSGSGSGTDFTFTISSLQPEDFATYYCQHYSTTPFTFGCGTKLEIK

SEQ ID NO: 46 - protein, 10 aa, Artificial Sequence
GGGGSGGGGS

SEQ ID NO: 47 - protein, 20 aa, Artificial Sequence
GGGGSGGGGSGGGGSGGGGS

SEQ ID NO: 48 - protein, 8 aa, Artificial Sequence
GFTFRTYG

SEQ ID NO: 49 - protein, 8 aa, Artificial Sequence
IWYDGSNK

SEQ ID NO: 50 - protein, 14 aa, Artificial Sequence
ARAPQWELVHEAFD

SEQ ID NO: 51 - protein, 6 aa, Artificial Sequence
NLGSKS

SEQ ID NO: 52 - protein, 11 aa, Artificial Sequence
QVWDSSSDHVV

SEQ ID NO: 53 - protein, 448 aa, Artificial Sequence
QMQLVESGGGVVQPGRSLRLSCAASGFTFRTYGMHWVRQAPGKGLEWVAVIWYDGSNKHYADSVKGRFTITRDNSKNTLNLQMNSLRAEDTAVYYCARAPQWELVHEAFDIWGQGTMVTVSSASTKGPSVFPLAPCSRSTSESTAALGCLVKDYFPEPVTVSWNSGALTSGVHTFPAVLQSSGLYSLSSVVTVPSSNFGTQTYTCNVDHKPSNTKVDKTVERKCCVECPPCPAPPVAGPSVFLFPPKPKDTLMISRTPEVTCVVVDVSHEDPEVQFNWYVDGVEVHNAKTKPREEQFNSTFRVVSVLTVVHQDWLNGKEYKCKVSNKGLPAPIEKTISKTKGQPREPQVYTLPPSREEMTKNQVSLTCLVKGFYPSDIAVEWESNGQPENNYKTTPPMLDSDGSFFLYSKLTVDKSRWQQGNVFSCSVMHEALHNHYTQKSLSLSPGK

SEQ ID NO: 54 - protein, 214 aa, Artificial Sequence
SYVLTQPPSVSVAPGQTARITCGGNNLGSKSVHWYQQKPGQAPVLVVYDDSDRPSWIPERFSGSNSGNTATLTISRGEAGDEADYYCQVWDSSSDHVVFGGGTKLTVLGQPKAAPSVTLFPPSSEELQANKATLVCLISDFYPGAVTVAWKADSSPVKAGVETTTPSKQSNNKYAASSYLSLTPEQWKSHRSYSCQVTHEGSTVEKTVAPTECS

SEQ ID NO: 55 - protein, 445 aa, Artificial Sequence
QVQLVQSGAEVKKPGASVKVSCKASGYTFTTYYIYWVRQAPGQGLEWMGGSNPSTGGTLDNEKFKTRVTMTVDKSTSTAYMELSSLRSEDTAVYYCTRSGRYAPFTYWGQGTLVTVSSASTKGPSVFPLAPCSRSTSESTAALGCLVKDYFPEPVTVSWNSGALTSGVHTFPAVLQSSGLYSLSSVVTVPSSSLGTKTYTCNVDHKPSNTKVDKRVESKYGPPCPPCPAPEFLGGPSVFLFPPKPKDTLMISRTPEVTCVVVDVSQEDPEVQFNWYVDGVEVHNAKTKPREEQFNSTYRVVSVLTVLHQDWLNGKEYKCKVSNKGLPSSIEKTISKAKGQPREPQVYTLPPSQEEMTKNQVSLTCLVKGFYPSDIAVEWESNGQPENNYKTTPPVLDSDGSFFLYSRLTVDKSRWQEGNVFSCSVMHEALHNHYTQKSLSLSLGK

SEQ ID NO: 56 - protein, 214 aa, Artificial Sequence
DIQMTQSPSSLSASVGDRVTITCKASQDVSTSVAWYQQKPGKAPKLLIYSASYRFTGVPSRFSGSGSGTDFTFTISSLQPEDFATYYCQHYSTTPFTFGQGTKLEIKRTVAAPSVFIFPPSDEQLKSGTASVVCLLNNFYPREAKVQWKVDNALQSGNSQESVTEQDSKDSTYSLSSTLTLSKADYEKHKVYACEVTHQGLSSPVTKSFNRGEC

SEQ ID NO: 57 - protein, 703 aa, Artificial Sequence
QMQLVESGGGVVQPGRSLRLSCAASGFTFRTYGMHWVRQAPGKGLEWVAVIWYDGSNKHYADSVKGRFTITRDNSKNTLNLQMNSLRAEDTAVYYCARAPQWELVHEAFDIWGQGTMVTVSSASTKGPSVFPLAPCSRSTSESTAALGCLVKDYFPEPVTVSWNSGALTSGVHTFPAVLQSSGLYSLSSVVTVPSSNFGTQTYTCNVDHKPSNTKVDKTVERKCCVECPPCPAPPVAGPSVFLFPPKPKDTLMISRTPEVTCVVVDVSHEDPEVQFNWYVDGVEVHNAKTKPREEQFNSTFRVVSVLTVVHQDWLNGKEYKCKVSNKGLPAPIEKTISKTKGQPREPQVYTLPPSREEMTKNQVSLTCLVKGFYPSDIAVEWESNGQPENNYKTTPPMLDSDGSFFLYSKLTVDKSRWQQGNVFSCSVMHEALHNHYTQKSLSLSPGKGGGGSGGGGSQVQLVQSGAEVKKPGASVKVSCKASGYTFTTYYIYWVRQAPGQCLEWMGGSNPSTGGTLDNEKFKTRVTMTVDKSTSTAYMELSSLRSEDTAVYYCTRSGRYAPFTYWGQGTLVTVSSGGGGSGGGGSGGGGSGGGGSDIQMTQSPSSLSASVGDRVTITCKASQDVSTSVAWYQQKPGKAPKLLIYSASYRFTGVPSRFSGSGSGTDFTFTISSLQPEDFATYYCQHYSTTPFTFGCGTKLEIK

SEQ ID NO: 58 - protein, 214 aa, Artificial Sequence; identical to SEQ ID NO: 54

SEQ ID NO: 59 - protein, 705 aa, Artificial Sequence
QVQLVQSGAEVKKPGASVKVSCKASGYTFTTYYIYWVRQAPGQGLEWMGGSNPSTGGTLDNEKFKTRVTMTVDKSTSTAYMELSSLRSEDTAVYYCTRSGRYAPFTYWGQGTLVTVSSASTKGPSVFPLAPCSRSTSESTAALGCLVKDYFPEPVTVSWNSGALTSGVHTFPAVLQSSGLYSLSSVVTVPSSSLGTKTYTCNVDHKPSNTKVDKRVESKYGPPCPPCPAPEFLGGPSVFLFPPKPKDTLMISRTPEVTCVVVDVSQEDPEVQFNWYVDGVEVHNAKTKPREEQFNSTYRVVSVLTVLHQDWLNGKEYKCKVSNKGLPSSIEKTISKAKGQPREPQVYTLPPSQEEMTKNQVSLTCLVKGFYPSDIAVEWESNGQPENNYKTTPPVLDSDGSFFLYSRLTVDKSRWQEGNVFSCSVMHEALHNHYTQKSLSLSLGKGGGGSGGGGSQMQLVESGGGVVQPGRSLRLSCAASGFTFRTYGMHWVRQAPGKCLEWVAVIWYDGSNKHYADSVKGRFTITRDNSKNTLNLQMNSLRAEDTAVYYCARAPQWELVHEAFDIWGQGTMVTVSSGGGGSGGGGSGGGGSGGGGSSYVLTQPPSVSVAPGQTARITCGGNNLGSKSVHWYQQKPGQAPVLVVYDDSDRPSWIPERFSGSNSGNTATLTISRGEAGDEADYYCQVWDSSSDHVVFGCGTKLTVL

SEQ ID NO: 60 - protein, 214 aa, Artificial Sequence; identical to SEQ ID NO: 56